European Patent Specification EP 4 017 870 B1, published July 30, 2025. Title: Compositions and Methods for Treating and Preventing Autoimmune Induced Cardiac Long QT Syndrome. Applicant: Boutjdir, Mohamed. The sequence listing filed with the application follows.

SEQUENCE LISTING (11 sequences)

SEQ ID NO: 1 - protein, 12 aa, Artificial Sequence
  Synthetic construct
GNMEQPHMDSRI

SEQ ID NO: 2 - protein, 7 aa, Artificial Sequence
  Synthetic construct
GWLHNLG

SEQ ID NO: 3 - protein, 12 aa, Artificial Sequence
  Synthetic construct
DQIGKPYNSSGL

SEQ ID NO: 4 - protein, 21 aa, Artificial Sequence
  Synthetic construct
GNMEQPHMDSRIGWLHNLGDQ

SEQ ID NO: 5 - protein, 15 aa, Artificial Sequence
  Synthetic construct
HMDSRIGWLHNLGDQ

SEQ ID NO: 6 - protein, 10 aa, Artificial Sequence
  Synthetic construct
IGKPYNSSGL

SEQ ID NO: 7 - protein, 16 aa, Artificial Sequence
  Synthetic construct
HNLGDQIGKPYNSSGL

SEQ ID NO: 8 - protein, 13 aa, Artificial Sequence
  Synthetic construct
GDQIGKPYNSSGL

SEQ ID NO: 9 - protein, 31 aa, Artificial Sequence
  Synthetic construct
GNMEQPHMDSRIGWLHNLGDQIGKPYNSSGL

SEQ ID NO: 10 - protein, 31 aa, Artificial Sequence
  Synthetic construct
NEQDRSGYHPMKWMSIILGGSGLNGPQNDLH

SEQ ID NO: 11 - protein, 94 aa, Artificial Sequence
  Synthetic construct
VSDVPTDLEVVAATPTSLLISWDAPAVTVRYYRITYGETGGNSPVQEFTVPGSKSTATISGLKPGVDYTITVYAVTGRGDSPASSKPISINYRT